European Patent Specification EP 3 310 932 B1, published August 30, 2023. Title: CRISPR/CAS9 COMPLEX FOR GENOMIC EDITING. Applicant: UAB Research Foundation Townes, Tim Ding, Lei Chang, Chia-Wei. The sequence listing filed with the application follows.

SEQUENCE LISTING (69 sequences)

SEQ ID NO: 1 - DNA, 19 bp, Artificial sequence
  Synthetic construct
taacggcagacttctccac

SEQ ID NO: 2 - DNA, 103 bp, Artificial sequence
  Synthetic construct
gtaacggcagacttctccacgttttagagctagaaatagcaagttaaaataaggctagtccgttatcaacttgaaaaagtggcaccgagtcggtgcttttttt

SEQ ID NO: 3 - protein, 1671 aa, Artificial sequence
  SEQ ID NO: 4
MDYKDHDGDYKDHDIDYKDDDDKMAPKKKRKVGIHGVPAADKKYSIGLDIGTNSVGWAVITDEYKVPSKKFKVLGNTDRHSIKKNLIGALLFDSGETAEATRLKRTARRRYTRRKNRICYLQEIFSNEMAKVDDSFFHRLEESFLVEEDKKHERHPIFGNIVDEVAYHEKYPTIYHLRKKLVDSTDKADLRLIYLALAHMIKFRGHFLIEGDLNPDNSDVDKLFIQLVQTYNQLFEENPINASGVDAKAILSARLSKSRRLENLIAQLPGEKKNGLFGNLIALSLGLTPNFKSNFDLAEDAKLQLSKDTYDDDLDNLLAQIGDQYADLFLAAKNLSDAILLSDILRVNTEITKAPLSASMIKRYDEHHQDLTLLKALVRQQLPEKYKEIFFDQSKNGYAGYIDGGASQEEFYKFIKPILEKMDGTEELLVKLNREDLLRKQRTFDNGSIPHQIHLGELHAILRRQEDFYPFLKDNREKIEKILTFRIPYYVGPLARGNSRFAWMTRKSEETITPWNFEEVVDKGASAQSFIERMTNFDKNLPNEKVLPKHSLLYEYFTVYNELTKVKYVTEGMRKPAFLSGEQKKAIVDLLFKTNRKVTVKQLKEDYFKKIECFDSVEISGVEDRFNASLGTYHDLLKIIKDKDFLDNEENEDILEDIVLTLTLFEDREMIEERLKTYAHLFDDKVMKQLKRRRYTGWGRLSRKLINGIRDKQSGKTILDFLKSDGFANRNFMQLIHDDSLTFKEDIQKAQVSGQGDSLHEHIANLAGSPAIKKGILQTVKVVDELVKVMGRHKPENIVIEMARENQTTQKGQKNSRERMKRIEEGIKELGSQILKEHPVENTQLQNEKLYLYYLQNGRDMYVDQELDINRLSDYDVDHIVPQSFLKDDSIDNKVLTRSDKNRGKSDNVPSEEVVKKMKNYWRQLLNAKLITQRKFDNLTKAERGGLSELDKAGFIKRQLVETRQITKHVAQILDSRMNTKYDENDKLIREVKVITLKSKLVSDFRKDFQFYKVREINNYHHAHDAYLNAVVGTALIKKYPKLESEFVYGDYKVYDVRKMIAKSEQEIGKATAKYFFYSNIMNFFKTEITLANGEIRKRPLIETNGETGEIVWDKGRDFATVRKVLSMPQVNIVKKTEVQTGGFSKESILPKRNSDKLIARKKDWDPKKYGGFDSPTVAYSVLVVAKVEKGKSKKLKSVKELLGITIMERSSFEKNPIDFLEAKGYKEVKKDLIIKLPKYSLFELENGRKRMLASAGELQKGNELALPSKYVNFLYLASHYEKLKGSPEDNEQKQLFVEQHKHYLDEIIEQISEFSKRVILADANLDKVLSAYNKHRDKPIREQAENIIHLFTLTNLGAPAAFKYFDTTIDRKRYTSTKEVLDATLIHQSITGLYETRIDLSQLGGDKRPAATKKAGQAKKKKGSGSNGSSGSASKGERLFRGKVPILVELKGDVNGHKFSVRGKGKGDATRGKLTLKFICTTGKLPVPWPTLVTTLTYGVQCFSRYPKHMKRHDFFKSAMPKGYVQERTISFKKDGKYKTRAEVKFEGRTLVNRIKLKGRDFKEKGNILGHKLRYNFNSHKVYITADKRKNGIKAKFKIRHNVKDGSVQLADHYQQNTPIGRGPVLLPRNHYLSTRSKLSKDPKEKRDHMVLLEFVTAAGIKHGRDERYK

SEQ ID NO: 4 - protein, 1720 aa, Artificial sequence
  Synthetic construct
YGRKKRRQRRRPPQAGGSMDYKDHDGDYKDHDIDYKDDDDKMAPKKKRKVGIHGVPAADKKYSIGLDIGTNSVGWAVITDEYKVPSKKFKVLGNTDRHSIKKNLIGALLFDSGETAEATRLKRTARRRYTRRKNRICYLQEIFSNEMAKVDDSFFHRLEESFLVEEDKKHERHPIFGNIVDEVAYHEKYPTIYHLRKKLVDSTDKADLRLIYLALAHMIKFRGHFLIEGDLNPDNSDVDKLFIQLVQTYNQLFEENPINASGVDAKAILSARLSKSRRLENLIAQLPGEKKNGLFGNLIALSLGLTPNFKSNFDLAEDAKLQLSKDTYDDDLDNLLAQIGDQYADLFLAAKNLSDAILLSDILRVNTEITKAPLSASMIKRYDEHHQDLTLLKALVRQQLPEKYKEIFFDQSKNGYAGYIDGGASQEEFYKFIKPILEKMDGTEELLVKLNREDLLRKQRTFDNGSIPHQIHLGELHAILRRQEDFYPFLKDNREKIEKILTFRIPYYVGPLARGNSRFAWMTRKSEETITPWNFEEVVDKGASAQSFIERMTNFDKNLPNEKVLPKHSLLYEYFTVYNELTKVKYVTEGMRKPAFLSGEQKKAIVDLLFKTNRKVTVKQLKEDYFKKIECFDSVEISGVEDRFNASLGTYHDLLKIIKDKDFLDNEENEDILEDIVLTLTLFEDREMIEERLKTYAHLFDDKVMKQLKRRRYTGWGRLSRKLINGIRDKQSGKTILDFLKSDGFANRNFMQLIHDDSLTFKEDIQKAQVSGQGDSLHEHIANLAGSPAIKKGILQTVKVVDELVKVMGRHKPENIVIEMARENQTTQKGQKNSRERMKRIEEGIKELGSQILKEHPVENTQLQNEKLYLYYLQNGRDMYVDQELDINRLSDYDVDHIVPQSFLKDDSIDNKVLTRSDKNRGKSDNVPSEEVVKKMKNYWRQLLNAKLITQRKFDNLTKAERGGLSELDKAGFIKRQLVETRQITKHVAQILDSRMNTKYDENDKLIREVKVITLKSKLVSDFRKDFQFYKVREINNYHHAHDAYLNAVVGTALIKKYPKLESEFVYGDYKVYDVRKMIAKSEQEIGKATAKYFFYSNIMNFFKTEITLANGEIRKRPLIETNGETGEIVWDKGRDFATVRKVLSMPQVNIVKKTEVQTGGFSKESILPKRNSDKLIARKKDWDPKKYGGFDSPTVAYSVLVVAKVEKGKSKKLKSVKELLGITIMERSSFEKNPIDFLEAKGYKEVKKDLIIKLPKYSLFELENGRKRMLASAGELQKGNELALPSKYVNFLYLASHYEKLKGSPEDNEQKQLFVEQHKHYLDEIIEQISEFSKRVILADANLDKVLSAYNKHRDKPIREQAENIIHLFTLTNLGAPAAFKYFDTTIDRKRYTSTKEVLDATLIHQSITGLYETRIDLSQLGGDKRPAATKKAGQAKKKKGSGSNGSSGSASKGERLFRGKVPILVELKGDVNGHKFSVRGKGKGDATRGKLTLKFICTTGKLPVPWPTLVTTLTYGVQCFSRYPKHMKRHDFFKSAMPKGYVQERTISFKKDGKYKTRAEVKFEGRTLVNRIKLKGRDFKEKGNILGHKLRYNFNSHKVYITADKRKNGIKAKFKIRHNVKDGSVQLADHYQQNTPIGRGPVLLPRNHYLSTRSKLSKDPKEKRDHMVLLEFVTAAGIKHGRDERYKGGSGGSVDGLFEAIEGFIENGWEGMIDGWYG

SEQ ID NO: 5 - DNA, 26 bp, Artificial sequence
  Synthetic construct
gctaattcactcccaaagaagacaag

SEQ ID NO: 6 - DNA, 20 bp, Synthetic construct
cttcagcaagccgagtcctg

SEQ ID NO: 7 - DNA, 60 bp, Artificial sequence
  Synthetic construct
gtcgacgtcgacgctcagtgaagctgaagtattccttctgcttcacagggcgaccactac

SEQ ID NO: 8 - DNA, 49 bp, Artificial sequence
  Synthetic construct
atttaaatcctcccctcgaacccttaccaaactcctatgcatactacag

SEQ ID NO: 9 - DNA, 60 bp, Artificial sequence
  Synthetic construct
ttaattaattaattagcattttaggttcaggttgtgagaacactagaagagaacaagtca

SEQ ID NO: 10 - DNA, 52 bp, Artificial sequence
  Synthetic construct
gtatacgtatacgcatacctggagaggggacaaggtcttgagatgcgagggt

SEQ ID NO: 11 - DNA, 52 bp, Artificial sequence
  Synthetic construct
agccaccttaattaagccaccatggcgcacgctgggagaacggggtacgata

SEQ ID NO: 12 - DNA, 60 bp, Synthetic construct
taacagagagaagttcgtggctccggatcccttgtggcccagataggcacccagggtgat

SEQ ID NO: 13 - DNA, 24 bp, Artificial sequence
  Synthetic construct
caccgtgagatacagatacagaca

SEQ ID NO: 14 - DNA, 24 bp, ARtificial sequence
  Synthetic construct
aaactgtctgtatctgtatctcac

SEQ ID NO: 15 - DNA, 25 bp, Artificial sequence
  Synthetic construct
aaacggcattccaggcaaatcattc

SEQ ID NO: 16 - DNA, 25 bp, Artificial sequence
  Synthetic construct
caccgcagcctaggcaaaggcctgc

SEQ ID NO: 17 - DNA, 25 bp, Artificial sequence
  Synthetic construct
aaacgcaggcctttgcctaggctgc

SEQ ID NO: 18 - DNA, 25 bp, Artificial sequence
  Synthetic construct
caccgtgccaacagaactgcctgat

SEQ ID NO: 19 - DNA, 25 bp, Artificial sequence
  Synthetic construct
aaacatcaggcagttctgttggcac

SEQ ID NO: 20 - DNA, 24 bp, Artificial sequence
  Synthetic construct
caccgaccagggtgcaagtgtgga

SEQ ID NO: 21 - DNA, 24 bp, Artificial sequence
  Synthetic construct
aaactccacacttgcaccctggtc

SEQ ID NO: 22 - DNA, 24 bp, Artificial sequence
  Synthetic construct
caccgctcctcagcctggcattca

SEQ ID NO: 23 - DNA, 24 bp, Artificial sequence
  Synthetic construct
aaactgaatgccaggctgaggagc

SEQ ID NO: 24 - DNA, 23 bp, Artificial sequence
  Synthetic construct
tgctaaagcgcatgctccagact

SEQ ID NO: 25 - DNA, 21 bp, Artificial sequence
  Synthetic construct
gtcttcatctcagggtcggct

SEQ ID NO: 26 - DNA, 21 bp, Artificial sequence
  Synthetic construct
cctctctgtgcattatggcag

SEQ ID NO: 27 - DNA, 19 bp, Artificial sequence
  Synthetic construct
gccttctatcgccttcttg

SEQ ID NO: 28 - DNA, 20 bp, Artificial sequence
  Synthetic construct
actcctccacctttgacgct

SEQ ID NO: 29 - DNA, 23 bp, Artificial sequence
  Synthetic construct
tcccctcttcaagggtctacatg

SEQ ID NO: 30 - DNA, 20 bp, Artificial sequence
  Synthetic construct
gtgcaaaatggaagggtttc

SEQ ID NO: 31 - DNA, 20 bp, Artificial sequence
  Synthetic construct
ggagctccgtgaagttgttc

SEQ ID NO: 32 - DNA, 21 bp, Artificial sequence
  Synthetic construct
tgtttcctttcactggccaca

SEQ ID NO: 33 - DNA, 21 bp, Artificial sequence
  Synthetic construct
aacggcaactggtgaacggta

SEQ ID NO: 34 - DNA, 22 bp, Artificial sequence
  Synthetic construct
ggcgatgccagaatagatgccg

SEQ ID NO: 35 - DNA, 29 bp, Artificial sequence
  Synthetic construct
ccaggccacttggctcctctatctccaga

SEQ ID NO: 36 - DNA, 25 bp, Artificial sequence
  Synthetic construct
ccttactgttgagactgcaatatcc

SEQ ID NO: 37 - DNA, 26 bp, Artificial sequence
  Synthetic construct
ctgaagtcccagtatatacttcacac

SEQ ID NO: 38 - DNA, 25 bp, Artificial sequence
  Synthetic construct
cccagaagcagtaataatcatcgag

SEQ ID NO: 39 - DNA, 23 bp, Artificial sequence
  Synthetic construct
atgtgggatgtagtagatcttgc

SEQ ID NO: 40 - DNA, 21 bp, Artificial sequence
  Synthetic construct
gggtcttacctcagcagttac

SEQ ID NO: 41 - DNA, 20 bp, Artificial sequence
  synthetic construct
cctcacacagtgtgacgcag

SEQ ID NO: 42 - DNA, 20 bp, Artificial sequence
  Synthetic construct
gactgagtacctgaaccggc

SEQ ID NO: 43 - DNA, 20 bp, Artificial sequence
  Synthetic construct
gggccaaactgagcagagtc

SEQ ID NO: 44 - DNA, 20 bp, Artificial sequence
  Synthetic construct
aagaccagggtggttgggac

SEQ ID NO: 45 - DNA, 20 bp, Artificial sequence
  Synthetic construct
gtaagaaaaatgcccacgtc

SEQ ID NO: 46 - DNA, 20 bp, Artifiical sequence
agtcagacgtctggagcttc

SEQ ID NO: 47 - DNA, 22 bp, Artificial sequence
  Synthetic construct
gtgagcagtgaaggcatgagtc

SEQ ID NO: 48 - DNA, 20 bp, Artificial sequence
  Synthetic construct
gtgagatacagatacagaca

SEQ ID NO: 49 - DNA, 20 bp, Artificial sequence
  Synthetic construct
aatgatttgcctggaatgcc

SEQ ID NO: 50 - protein, 23 aa, Artificial sequence
  Synthetic construct
GLFEAIEGFIENGWEGMIDGWYG

SEQ ID NO: 51 - protein, 14 aa, Artificial sequence
  Synthetic construct
YGRKKRRQRRRPPQ

SEQ ID NO: 52 - DNA, 91 bp, Artificial sequence
  Synthetic construct
atccacgttcaccttgccccacagggcagtaacggcagacttctcctcaggagtcaggtgcaccatggtgtctgtttgaggttgctagtga

SEQ ID NO: 53 - DNA, 95 bp, Artificial sequence
  Synthetic construct
cttcatccacgttcaccttgccccacagggcagtaacggcagatttttcctcaggagtcaggtgcaccatggtgtctgtttgaggttgctagtga

SEQ ID NO: 54 - DNA, 39 bp, Artificial sequence
  Synthetic construct
taatacgactcactatagggtaacggcagacttctccac

SEQ ID NO: 55 - DNA, 21 bp, Artificial sequence
  Synthetic construct
aaaaagcaccgactcggtgcc

SEQ ID NO: 56 - DNA, 14 bp, Artificial sequence
  Synthetic construct
tcctgaggaaaaat

SEQ ID NO: 57 - DNA, 16 bp, Artificial sequence
  Synthetic construct
tgactcctgaggagaa

SEQ ID NO: 58 - DNA, 15 bp, Artificial sequence
  Synthetic construct
actcctgtggagaag

SEQ ID NO: 59 - DNA, 25 bp, Artificial sequence
  Synthetic construct
cagagccatctattgcttacatttg

SEQ ID NO: 60 - DNA, 20 bp, Artificial sequence
  Synthetic construct
ggcctcaccaccaacttcat

SEQ ID NO: 61 - protein, 60 aa, Artificial sequence
  Synthetic construct
YGRKKRRQRRRPPQAGGGSGGSYGRKKRRQRRRPPQAGGGSGGSYGRKKRRQRRRPPQAG

SEQ ID NO: 62 - RNA, 104 nt, Artificial sequence
  Synthetic construct
gggucugccguuacugcccugguuuuagagcuagaaauagcaaguuaaaauaaggcuaguccguuaucaacuugaaaaaguggcaccgagucggugcuuuuuuu

SEQ ID NO: 63 - RNA, 105 nt, Artificial sequence
  Synthetic construct
ggguaacggcagacuucuccacguuuuagagcuagaaauagcaaguuaaaauaaggcuaguccguuaucaacuugaaaaaguggcaccgagucggugcuuuuuuu

SEQ ID NO: 64 - DNA, 90 bp, Artificial sequence
  Synthetic construct
acctcaaacagacaccatggtgcacctgactcctgaggagaagtctgccgtcacagctctgtggggcaaggtgaacgtggatgaagttgg

SEQ ID NO: 65 - DNA, 38 bp, Artificial sequence
  Synthetic construct
taatacgactcactatagggtctgccgttactgccctg

SEQ ID NO: 66 - DNA, 20 bp, Artificial sequence
  Synthetic construct
tccacatgcccagtttctat

SEQ ID NO: 67 - DNA, 25 bp, Artificial sequence
  Synthetic construct
agtagcaatttgtactgatggtatg

SEQ ID NO: 68 - DNA, 20 bp, Artificial sequence
  Synthetic construct
ggtctgccgttactgccctg

SEQ ID NO: 69 - DNA, 20 bp, Artificial sequence
  Synthetic construct
gtaacggcagacttctccac